European Patent Application EP 4 170 044 A1, published April 26, 2023. Title: METHOD FOR IDENTIFICATION AND ENUMERATION OF NUCLEIC ACID SEQUENCE, EXPRESSION, COPY, OR DNA METHYLATION CHANGES USING COMBINED NUCLEASE, LIGASE, POLYMERASE, AND SEQUENCING REACTIONS. Applicant: Cornell University. Application EP. The sequence listing filed with the application follows.

SEQUENCE LISTING (157 sequences)

SEQ ID NO: 1 - DNA, 33 bp, synthetic construct
  misc_feature 1..33: note = Primer
  source 1..33: mol_type = other DNA
acactctttccctacacgacgctcttccgatct

SEQ ID NO: 2 - DNA, 33 bp, synthetic construct
  misc_feature 1..33: note = Primer
  source 1..33: mol_type = other DNA
gatcggaagagcacacgtctgaactccagtcac

SEQ ID NO: 3 - DNA, 29 bp, synthetic construct
  misc_feature 1..29: note = Primer
  source 1..29: mol_type = other DNA
aatgatacggcgaccaccgagatctacac

SEQ ID NO: 4 - DNA, 34 bp, synthetic construct
  misc_feature 1..34: note = Primer
  source 1..34: mol_type = other DNA
gtgactggagttcagacgtgtgctcttccgatct

SEQ ID NO: 5 - DNA, 30 bp, synthetic construct
  misc_feature 1..30: note = Primer
  source 1..30: mol_type = other DNA
  misc_feature <1: note = 5SpC3 C3 spacer
aaaaaaaaaaaaaaaaaaaaaaaaaaaaaa

SEQ ID NO: 6 - DNA, 14 bp, synthetic construct
  misc_feature 1..14: note = Short linker T Overhang
  source 1..14: mol_type = other DNA
  misc_feature 3..4: note = thiophosphate backbone
tgctcttccgatct

SEQ ID NO: 7 - DNA, 12 bp, synthetic construct
  misc_feature 1..12: note = Bottom linker T overhang
  source 1..12: mol_type = other DNA
  misc_feature 10..11: note = thiophosphate backbone
gatcggaagagc

SEQ ID NO: 8 - DNA, 13 bp, synthetic construct
  misc_feature 1..13: note = Short linker blunt end
  source 1..13: mol_type = other DNA
agatcggaagagc

SEQ ID NO: 9 - DNA, 18 bp, synthetic construct
  misc_feature 1..18: note = Medium linker T overhang
  source 1..18: mol_type = other DNA
  misc_feature 3..4: note = thiophosphate backbone
tcgacgctcttccgatct

SEQ ID NO: 10 - DNA, 16 bp, synthetic construct
  misc_feature 1..16: note = Medium linker T overhang
  source 1..16: mol_type = other DNA
  misc_feature 14..15: note = thiophosphate backbone
gatcggaagagcacac

SEQ ID NO: 11 - DNA, 29 bp, synthetic construct
  misc_feature 1..29: note = Primer
  modified_base 10: mod_base = OTHER; note = Deoxyuridine
  modified_base 15: mod_base = OTHER; note = Deoxyuridine
  source 1..29: mol_type = other DNA
aggcaagagngcctngacgatacagctaa

SEQ ID NO: 12 - DNA, 59 bp, synthetic construct
  misc_feature 1..59: note = Primer
  modified_base 40: mod_base = OTHER; note = Deoxyuridine
  modified_base 45: mod_base = OTHER; note = Deoxyuridine
  source 1..59: mol_type = other DNA
  misc_feature <1: note = 5SpC3 C3 spacer
aaaaaaaaaaaaaaaaaaaaaaaaaaaaaaaggcaagagngcctngacgatacagctaa

SEQ ID NO: 13 - DNA, 84 bp, synthetic construct
  misc_feature 1..84: note = Primer
  source 1..84: mol_type = other DNA
aggcaagagtgccttgacgatacagctaattcagaatcattttgtggacgagatcggaagagcacacgtctgaactccagtcac

SEQ ID NO: 14 - DNA, 77 bp, synthetic construct
  misc_feature 1..77: note = Primer
  modified_base 42: mod_base = OTHER; note = Deoxyuridine
  modified_base 50: mod_base = OTHER; note = Deoxyuridine
  modified_base 64: mod_base = OTHER; note = Deoxyuridine
  modified_base 73: mod_base = OTHER; note = Deoxyuridine
  source 1..77: mol_type = other DNA
gagcacacgtctgaactccagtcaccgagtaatatctcgtangccgtctnctgcttgacacacncgcaatganacgg

SEQ ID NO: 15 - DNA, 78 bp, synthetic construct
  misc_feature 1..78: note = Primer
  modified_base 42: mod_base = OTHER; note = Deoxyuridine
  modified_base 55: mod_base = OTHER; note = Deoxyuridine
  modified_base 67: mod_base = OTHER; note = Deoxyuridine
  source 1..78: mol_type = other DNA
gagcgtcgtgtagggaaagagtgtaggctatagtgtagatcncggtggtcgccgnatcattgcgagngtgtcaagcag

SEQ ID NO: 16 - DNA, 83 bp, synthetic construct
  misc_feature 1..83: note = Primer
  source 1..83: mol_type = other DNA
acactctttccctacacgacgctcttccgatctttattataaggcctgctgaaaatgactgaatataaacttgtggtagttgg

SEQ ID NO: 17 - DNA, 37 bp, synthetic construct
  misc_feature 1..37: note = Primer
  modified_base 15: mod_base = OTHER; note = Deoxyuridine
  modified_base 22: mod_base = OTHER; note = Deoxyuridine
  source 1..37: mol_type = other DNA
ccaactaccacaagnttatatncagtcattttcagca

SEQ ID NO: 18 - DNA, 67 bp, synthetic construct
  misc_feature 1..67: note = Primer
  modified_base 45: mod_base = OTHER; note = Deoxyuridine
  modified_base 52: mod_base = OTHER; note = Deoxyuridine
  source 1..67: mol_type = other DNA
  misc_feature <1: note = 5SpC3 C3 spacer
aaaaaaaaaaaaaaaaaaaaaaaaaaaaaaccaactaccacaagnttatatncagtcattttcagca

SEQ ID NO: 19 - DNA, 30 bp, synthetic construct
  misc_feature 1..30: note = Primer
  modified_base 11: mod_base = OTHER; note = Deoxyuridine
  modified_base 20: mod_base = OTHER; note = Deoxyuridine
  source 1..30: mol_type = other DNA
ctcgatggagngggtcccancagtttgaac

SEQ ID NO: 20 - DNA, 60 bp, synthetic construct
  misc_feature 1..60: note = Primer
  modified_base 41: mod_base = OTHER; note = Deoxyuridine
  modified_base 50: mod_base = OTHER; note = Deoxyuridine
  source 1..60: mol_type = other DNA
  misc_feature <1: note = 5SpC3 C3 spacer
aaaaaaaaaaaaaaaaaaaaaaaaaaaaaactcgatggagngggtcccancagtttgaac

SEQ ID NO: 21 - DNA, 84 bp, synthetic construct
  misc_feature 1..84: note = Primer
  source 1..84: mol_type = other DNA
ctcgatggagtgggtcccatcagtttgaacagttgtctggatccattttgagatcggaagagcacacgtctgaactccagtcac

SEQ ID NO: 22 - DNA, 83 bp, synthetic construct
  misc_feature 1..83: note = Primer
  source 1..83: mol_type = other DNA
acactctttccctacacgacgctcttccgatcttttcttcatgaagacctcacagtaaaaataggtgattttggtctagctac

SEQ ID NO: 23 - DNA, 41 bp, synthetic construct
  misc_feature 1..41: note = Primer
  modified_base 16: mod_base = OTHER; note = Deoxyuridine
  modified_base 27: mod_base = OTHER; note = Deoxyuridine
  source 1..41: mol_type = other DNA
gtagctagaccaaaancacctattttnactgtgaggtcttc

SEQ ID NO: 24 - DNA, 71 bp, synthetic construct
  misc_feature 1..71: note = Primer
  modified_base 46: mod_base = OTHER; note = Deoxyuridine
  modified_base 57: mod_base = OTHER; note = Deoxyuridine
  source 1..71: mol_type = other DNA
  misc_feature <1: note = 5SpC3 C3 spacer
aaaaaaaaaaaaaaaaaaaaaaaaaaaaaagtagctagaccaaaancacctattttnactgtgaggtcttc

SEQ ID NO: 25 - DNA, 25 bp, synthetic construct
  misc_feature 1..25: note = Primer
  modified_base 10: mod_base = OTHER; note = Deoxyuridine
  modified_base 18: mod_base = OTHER; note = Deoxyuridine
  source 1..25: mol_type = other DNA
gtgcagctgngggttgantccacac

SEQ ID NO: 26 - DNA, 55 bp, synthetic construct
  misc_feature 1..55: note = Primer
  modified_base 40: mod_base = OTHER; note = Deoxyuridine
  modified_base 48: mod_base = OTHER; note = Deoxyuridine
  source 1..55: mol_type = other DNA
  misc_feature <1: note = 5SpC3 C3 spacer
aaaaaaaaaaaaaaaaaaaaaaaaaaaaaagtgcagctgngggttgantccacac

SEQ ID NO: 27 - DNA, 83 bp, synthetic construct
  misc_feature 1..83: note = Primer
  source 1..83: mol_type = other DNA
gtgcagctgtgggttgattccacacccccgcccggcacccgcgtccgcgagatcggaagagcacacgtctgaactccagtcac

SEQ ID NO: 28 - DNA, 83 bp, synthetic construct
  misc_feature 1..83: note = Primer
  source 1..83: mol_type = other DNA
acactctttccctacacgacgctcttccgatcttcctacagtactcccctgccctcaacaagatgttttgccaactggccaag

SEQ ID NO: 29 - DNA, 29 bp, synthetic construct
  misc_feature 1..29: note = Primer
  modified_base 11: mod_base = OTHER; note = Deoxyuridine
  modified_base 21: mod_base = OTHER; note = Deoxyuridine
  source 1..29: mol_type = other DNA
cttggccagtnggcaaaacancttgttga

SEQ ID NO: 30 - DNA, 59 bp, synthetic construct
  misc_feature 1..59: note = Primer
  modified_base 41: mod_base = OTHER; note = Deoxyuridine
  modified_base 51: mod_base = OTHER; note = Deoxyuridine
  source 1..59: mol_type = other DNA
  misc_feature <1: note = 5SpC3 C3 spacer
aaaaaaaaaaaaaaaaaaaaaaaaaaaaaacttggccagtnggcaaaacancttgttga

SEQ ID NO: 31 - DNA, 26 bp, synthetic construct
  misc_feature 1..26: note = Primer
  modified_base 10: mod_base = OTHER; note = Deoxyuridine
  modified_base 15: mod_base = OTHER; note = Deoxyuridine
  source 1..26: mol_type = other DNA
gagcgctgcncaganagcgatggtga

SEQ ID NO: 32 - DNA, 56 bp, synthetic construct
  misc_feature 1..56: note = Primer
  modified_base 40: mod_base = OTHER; note = Deoxyuridine
  modified_base 45: mod_base = OTHER; note = Deoxyuridine
  source 1..56: mol_type = other DNA
  misc_feature <1: note = 5SpC3 C3 spacer
aaaaaaaaaaaaaaaaaaaaaaaaaaaaaagagcgctgcncaganagcgatggtga

SEQ ID NO: 33 - DNA, 84 bp, synthetic construct
  misc_feature 1..84: note = Primer
  source 1..84: mol_type = other DNA
gagcgctgctcagatagcgatggtgagcagctggagctggagagacgacaagatcggaagagcacacgtctgaactccagtcac

SEQ ID NO: 34 - DNA, 83 bp, synthetic construct
  misc_feature 1..83: note = Primer
  source 1..83: mol_type = other DNA
acactctttccctacacgacgctcttccgatcttccgcgccatggccatctacaagcagtcacagcacatgacggaggttgtg

SEQ ID NO: 35 - DNA, 27 bp, synthetic construct
  misc_feature 1..27: note = Primer
  modified_base 12: mod_base = OTHER; note = Deoxyuridine
  modified_base 20: mod_base = OTHER; note = Deoxyuridine
  source 1..27: mol_type = other DNA
cacaacctccgncatgtgcngtgactg

SEQ ID NO: 36 - DNA, 57 bp, synthetic construct
  misc_feature 1..57: note = Primer
  modified_base 42: mod_base = OTHER; note = Deoxyuridine
  modified_base 50: mod_base = OTHER; note = Deoxyuridine
  source 1..57: mol_type = other DNA
  misc_feature <1: note = 5SpC3 C3 spacer
aaaaaaaaaaaaaaaaaaaaaaaaaaaaaacacaacctccgncatgtgcngtgactg

SEQ ID NO: 37 - DNA, 31 bp, synthetic construct
  misc_feature 1..31: note = Primer
  modified_base 11: mod_base = OTHER; note = Deoxyuridine
  modified_base 22: mod_base = OTHER; note = Deoxyuridine
  source 1..31: mol_type = other DNA
gaaacactttncgacatagtgnggtggtgcc

SEQ ID NO: 38 - DNA, 61 bp, synthetic construct
  misc_feature 1..61: note = Primer
  modified_base 41: mod_base = OTHER; note = Deoxyuridine
  modified_base 52: mod_base = OTHER; note = Deoxyuridine
  source 1..61: mol_type = other DNA
  misc_feature <1: note = 5SpC3 C3 spacer
aaaaaaaaaaaaaaaaaaaaaaaaaaaaaagaaacactttncgacatagtgnggtggtgcc

SEQ ID NO: 39 - DNA, 84 bp, synthetic construct
  misc_feature 1..84: note = Primer
  source 1..84: mol_type = other DNA
gaaacacttttcgacatagtgtggtggtgccctatgagccgcctgaggtcagatcggaagagcacacgtctgaactccagtcac

SEQ ID NO: 40 - DNA, 83 bp, synthetic construct
  misc_feature 1..83: note = Primer
  source 1..83: mol_type = other DNA
acactctttccctacacgacgctcttccgatctggcccctcctcagcatcttatccgagtggaaggaaatttgcgtgtggagt

SEQ ID NO: 41 - DNA, 27 bp, synthetic construct
  misc_feature 1..27: note = Primer
  modified_base 15: mod_base = OTHER; note = Deoxyuridine
  modified_base 20: mod_base = OTHER; note = Deoxyuridine
  source 1..27: mol_type = other DNA
actccacacgcaaanttccntccactc

SEQ ID NO: 42 - DNA, 57 bp, synthetic construct
  misc_feature 1..57: note = Primer
  modified_base 45: mod_base = OTHER; note = Deoxyuridine
  modified_base 50: mod_base = OTHER; note = Deoxyuridine
  source 1..57: mol_type = other DNA
  misc_feature <1: note = 5SpC3 C3 spacer
aaaaaaaaaaaaaaaaaaaaaaaaaaaaaaactccacacgcaaanttccntccactc

SEQ ID NO: 43 - DNA, 28 bp, synthetic construct
  misc_feature 1..28: note = Primer
  modified_base 12: mod_base = OTHER; note = Deoxyuridine
  modified_base 18: mod_base = OTHER; note = Deoxyuridine
  source 1..28: mol_type = other DNA
cctcaccatcancacacnggaagactcc

SEQ ID NO: 44 - DNA, 58 bp, synthetic construct
  misc_feature 1..58: note = Primer
  modified_base 42: mod_base = OTHER; note = Deoxyuridine
  modified_base 48: mod_base = OTHER; note = Deoxyuridine
  source 1..58: mol_type = other DNA
  misc_feature <1: note = 5SpC3 C3 spacer
aaaaaaaaaaaaaaaaaaaaaaaaaaaaaacctcaccatcancacacnggaagactcc

SEQ ID NO: 45 - DNA, 84 bp, synthetic construct
  misc_feature 1..84: note = Primer
  source 1..84: mol_type = other DNA
cctcaccatcatcacactggaagactccaggtcaggagccacttgccaccagatcggaagagcacacgtctgaactccagtcac

SEQ ID NO: 46 - DNA, 83 bp, synthetic construct
  misc_feature 1..83: note = Primer
  source 1..83: mol_type = other DNA
acactctttccctacacgacgctcttccgatctgctctgactgtaccaccatccactacaactacatgtgtaacagttcctgc

SEQ ID NO: 47 - DNA, 34 bp, synthetic construct
  misc_feature 1..34: note = Primer
  modified_base 12: mod_base = OTHER; note = Deoxyuridine
  modified_base 20: mod_base = OTHER; note = Deoxyuridine
  source 1..34: mol_type = other DNA
gcaggaactgtnacacatgnagttgtagtggatg

SEQ ID NO: 48 - DNA, 64 bp, synthetic construct
  misc_feature 1..64: note = Primer
  modified_base 42: mod_base = OTHER; note = Deoxyuridine
  modified_base 50: mod_base = OTHER; note = Deoxyuridine
  source 1..64: mol_type = other DNA
  misc_feature <1: note = 5SpC3 C3 spacer
aaaaaaaaaaaaaaaaaaaaaaaaaaaaaagcaggaactgtnacacatgnagttgtagtggatg

SEQ ID NO: 49 - DNA, 24 bp, synthetic construct
  misc_feature 1..24: note = Primer
  modified_base 15: mod_base = OTHER; note = Deoxyuridine
  source 1..24: mol_type = other DNA
gggagagaccggcgnacagaggaa

SEQ ID NO: 50 - DNA, 54 bp, synthetic construct
  misc_feature 1..54: note = Primer
  modified_base 45: mod_base = OTHER; note = Deoxyuridine
  source 1..54: mol_type = other DNA
  misc_feature <1: note = 5SpC3 C3 spacer
aaaaaaaaaaaaaaaaaaaaaaaaaaaaaagggagagaccggcgnacagaggaa

SEQ ID NO: 51 - DNA, 84 bp, synthetic construct
  misc_feature 1..84: note = Primer
  modified_base 15: mod_base = OTHER; note = Deoxyuridine
  source 1..84: mol_type = other DNA
gggagagaccggcgnacagaggaagagaatctccgcaagaaaggagagccagatcggaagagcacacgtctgaactccagtcac

SEQ ID NO: 52 - DNA, 83 bp, synthetic construct
  misc_feature 1..83: note = Primer
  source 1..83: mol_type = other DNA
acactctttccctacacgacgctcttccgatctctcttttcctatcctgagtagtggtaatctactgggacggaacagctttg

SEQ ID NO: 53 - DNA, 28 bp, synthetic construct
  misc_feature 1..28: note = Primer
  modified_base 7: mod_base = OTHER; note = Deoxyuridine
  modified_base 14: mod_base = OTHER; note = Deoxyuridine
  source 1..28: mol_type = other DNA
caaagcngttccgncccagtagattacc

SEQ ID NO: 54 - DNA, 58 bp, synthetic construct
  misc_feature 1..58: note = Primer
  modified_base 37: mod_base = OTHER; note = Deoxyuridine
  modified_base 44: mod_base = OTHER; note = Deoxyuridine
  source 1..58: mol_type = other DNA
  misc_feature <1: note = 5SpC3 C3 spacer
aaaaaaaaaaaaaaaaaaaaaaaaaaaaaacaaagcngttccgncccagtagattacc

SEQ ID NO: 55 - DNA, 25 bp, synthetic construct
  misc_feature 1..25: note = Primer
  modified_base 12: mod_base = OTHER; note = Deoxyuridine
  modified_base 17: mod_base = OTHER; note = Deoxyuridine
  source 1..25: mol_type = other DNA
gtaggcaagagngcttngacgatac

SEQ ID NO: 56 - DNA, 55 bp, synthetic construct
  misc_feature 1..55: note = Primer
  modified_base 42: mod_base = OTHER; note = Deoxyuridine
  modified_base 47: mod_base = OTHER; note = Deoxyuridine
  source 1..55: mol_type = other DNA
  misc_feature <1: note = 5SpC3 C3 spacer
aaaaaaaaaaaaaaaaaaaaaaaaaaaaaagtaggcaagagngcttngacgatac

SEQ ID NO: 57 - DNA, 119 bp, synthetic construct
  misc_feature 1..119: note = Primer
  misc_feature 81..85: note = n is a, c, g, or t
  source 1..119: mol_type = other DNA
gtaggcaagagtgctttgacgatacagctgattcagaatcatttcgtggacgaatatgacccaacaatagaggtagatctnnnnnagatcggaagagcacacgtctgaactccagtcac

SEQ ID NO: 58 - DNA, 77 bp, synthetic construct
  misc_feature 1..77: note = Primer
  modified_base 42: mod_base = OTHER; note = Deoxyuridine
  modified_base 50: mod_base = OTHER; note = Deoxyuridine
  modified_base 64: mod_base = OTHER; note = Deoxyuridine
  modified_base 73: mod_base = OTHER; note = Deoxyuridine
  source 1..77: mol_type = other DNA
gagcacacgtctgaactccagtcacttctgaatatctcgtangccgtctnctgcttgacacacncgcaatganacgg

SEQ ID NO: 59 - DNA, 78 bp, synthetic construct
  misc_feature 1..78: note = Primer
  modified_base 42: mod_base = OTHER; note = Deoxyuridine
  modified_base 55: mod_base = OTHER; note = Deoxyuridine
  modified_base 67: mod_base = OTHER; note = Deoxyuridine
  source 1..78: mol_type = other DNA
gagcgtcgtgtagggaaagagtgtgcctctatgtgtagatcncggtggtcgccgnatcattgcgagngtgtcaagcag

SEQ ID NO: 60 - DNA, 118 bp, synthetic construct
  misc_feature 1..118: note = Primer
  misc_feature 34..38: note = n is a, c, g, or t
  source 1..118: mol_type = other DNA
acactctttccctacacgacgctcttccgatctnnnnnctaatatggtcacattttcattgtttttattataaggtctgctgaaaatgaccgaatataaacttgtagtagttggagct

SEQ ID NO: 61 - DNA, 31 bp, synthetic construct
  misc_feature 1..31: note = Primer
  modified_base 10: mod_base = OTHER; note = Deoxyuridine
  modified_base 20: mod_base = OTHER; note = Deoxyuridine
  source 1..31: mol_type = other DNA
agctccaacnactacaagtntatattcggtc

SEQ ID NO: 62 - DNA, 61 bp, synthetic construct
  misc_feature 1..61: note = Primer
  modified_base 40: mod_base = OTHER; note = Deoxyuridine
  modified_base 50: mod_base = OTHER; note = Deoxyuridine
  source 1..61: mol_type = other DNA
  misc_feature <1: note = 5SpC3 C3 spacer
aaaaaaaaaaaaaaaaaaaaaaaaaaaaaaagctccaacnactacaagtntatattcggtc

SEQ ID NO: 63 - DNA, 21 bp, synthetic construct
  misc_feature 1..21: note = Primer
  modified_base 4: mod_base = OTHER; note = Deoxyuridine
  modified_base 10: mod_base = OTHER; note = Deoxyuridine
  source 1..21: mol_type = other DNA
aaanctcganggagcgggtcc

SEQ ID NO: 64 - DNA, 51 bp, synthetic construct
  misc_feature 1..51: note = Primer
  modified_base 34: mod_base = OTHER; note = Deoxyuridine
  modified_base 40: mod_base = OTHER; note = Deoxyuridine
  source 1..51: mol_type = other DNA
  misc_feature <1: note = 5SpC3 C3 spacer
aaaaaaaaaaaaaaaaaaaaaaaaaaaaaaaaanctcganggagcgggtcc

SEQ ID NO: 65 - DNA, 119 bp, synthetic construct
  misc_feature 1..119: note = Primer
  misc_feature 81..85: note = n is a, c, g, or t
  source 1..119: mol_type = other DNA
aaatctcgatggagcgggtcccatcagttcgaacagttgtctgggtccattttgtggatagtaagaattgaggctgttttnnnnnagatcggaagagcacacgtctgaactccagtcac

SEQ ID NO: 66 - DNA, 118 bp, synthetic construct
  misc_feature 1..118: note = Primer
  misc_feature 34..38: note = n is a, c, g, or t
  source 1..118: mol_type = other DNA
acactctttccctacacgacgctcttccgatctnnnnntttccttcacttactacacctcggatatatttcttcacgaagacctcacagtgaaaataggtgatttcggtctagctaca

SEQ ID NO: 67 - DNA, 30 bp, synthetic construct
  misc_feature 1..30: note = Primer
  modified_base 7: mod_base = OTHER; note = Deoxyuridine
  modified_base 17: mod_base = OTHER; note = Deoxyuridine
  source 1..30: mol_type = other DNA
tgtagcnagaccgaaancacctattttcac

SEQ ID NO: 68 - DNA, 60 bp, synthetic construct
  misc_feature 1..60: note = Primer
  modified_base 37: mod_base = OTHER; note = Deoxyuridine
  modified_base 47: mod_base = OTHER; note = Deoxyuridine
  source 1..60: mol_type = other DNA
  misc_feature <1: note = 5SpC3 C3 spacer
aaaaaaaaaaaaaaaaaaaaaaaaaaaaaatgtagcnagaccgaaancacctattttcac

SEQ ID NO: 69 - DNA, 18 bp, synthetic construct
  misc_feature 1..18: note = Primer
  modified_base 7: mod_base = OTHER; note = Deoxyuridine
  modified_base 15: mod_base = OTHER; note = Deoxyuridine
  source 1..18: mol_type = other DNA
aggcgcngcccccancat

SEQ ID NO: 70 - DNA, 48 bp, synthetic construct
  misc_feature 1..48: note = Primer
  modified_base 37: mod_base = OTHER; note = Deoxyuridine
  modified_base 45: mod_base = OTHER; note = Deoxyuridine
  source 1..48: mol_type = other DNA
  misc_feature <1: note = 5SpC3 C3 spacer
aaaaaaaaaaaaaaaaaaaaaaaaaaaaaaaggcgcngcccccancat

SEQ ID NO: 71 - DNA, 119 bp, synthetic construct
  misc_feature 1..119: note = Primer
  misc_feature 81..85: note = n is a, c, g, or t
  source 1..119: mol_type = other DNA
aggcgctgcccccatcatgagcgctgctcggatagcgatggtgaacagctggagctggaaagacgacagggctggctgccnnnnnagatcggaagagcacacgtctgaactccagtcac

SEQ ID NO: 72 - DNA, 118 bp, synthetic construct
  misc_feature 1..118: note = Primer
  misc_feature 34..38: note = n is a, c, g, or t
  source 1..118: mol_type = other DNA
acactctttccctacacgacgctcttccgatctnnnnntgtgggtcgattccacacccccacccggcacccgcgttcgcgccatggccatttacaagcagtcacaacacatgacggag

SEQ ID NO: 73 - DNA, 29 bp, synthetic construct
  misc_feature 1..29: note = Primer
  modified_base 11: mod_base = OTHER; note = Deoxyuridine
  modified_base 20: mod_base = OTHER; note = Deoxyuridine
  source 1..29: mol_type = other DNA
ctccgtcatgngttgtgacngcttgtaaa

SEQ ID NO: 74 - DNA, 59 bp, synthetic construct
  misc_feature 1..59: note = Primer
  modified_base 41: mod_base = OTHER; note = Deoxyuridine
  modified_base 50: mod_base = OTHER; note = Deoxyuridine
  source 1..59: mol_type = other DNA
  misc_feature <1: note = 5SpC3 C3 spacer
aaaaaaaaaaaaaaaaaaaaaaaaaaaaaactccgtcatgngttgtgacngcttgtaaa

SEQ ID NO: 75 - DNA, 26 bp, synthetic construct
  misc_feature 1..26: note = Primer
  modified_base 8: mod_base = OTHER; note = Deoxyuridine
  modified_base 18: mod_base = OTHER; note = Deoxyuridine
  source 1..26: mol_type = other DNA
aacacttntcgacacagngtggtggt

SEQ ID NO: 76 - DNA, 56 bp, synthetic construct
  misc_feature 1..56: note = Primer
  modified_base 38: mod_base = OTHER; note = Deoxyuridine
  modified_base 48: mod_base = OTHER; note = Deoxyuridine
  source 1..56: mol_type = other DNA
  misc_feature <1: note = 5SpC3 C3 spacer
aaaaaaaaaaaaaaaaaaaaaaaaaaaaaaaacacttntcgacacagngtggtggt

SEQ ID NO: 77 - DNA, 119 bp, synthetic construct
  misc_feature 1..119: note = Primer
  misc_feature 81..85: note = n is a, c, g, or t
  source 1..119: mol_type = other DNA
aacacttttcgacacagtgtggtggtgccttatgagccgcctgaagtctggtttgcaaccggagtctctgggaggaagggnnnnnagatcggaagagcacacgtctgaactccagtcac

SEQ ID NO: 78 - DNA, 118 bp, synthetic construct
  misc_feature 1..118: note = Primer
  misc_feature 34..38: note = n is a, c, g, or t
  source 1..118: mol_type = other DNA
acactctttccctacacgacgctcttccgatctnnnnnctcactgactgctcttaggtctagcccctcctcagcaccttatccgagtggagggaaatttgcgtgtagagtatttggat

SEQ ID NO: 79 - DNA, 31 bp, synthetic construct
  misc_feature 1..31: note = Primer
  modified_base 11: mod_base = OTHER; note = Deoxyuridine
  modified_base 23: mod_base = OTHER; note = Deoxyuridine
  source 1..31: mol_type = other DNA
atccaaatacnctacacgcaaanttccctcc

SEQ ID NO: 80 - DNA, 61 bp, synthetic construct
  misc_feature 1..61: note = Primer
  modified_base 41: mod_base = OTHER; note = Deoxyuridine
  modified_base 53: mod_base = OTHER; note = Deoxyuridine
  source 1..61: mol_type = other DNA
  misc_feature <1: note = 5SpC3 C3 spacer
aaaaaaaaaaaaaaaaaaaaaaaaaaaaaaatccaaatacnctacacgcaaanttccctcc

SEQ ID NO: 81 - DNA, 21 bp, synthetic construct
  misc_feature 1..21: note = Primer
  modified_base 8: mod_base = OTHER; note = Deoxyuridine
  source 1..21: mol_type = other DNA
ggcggcangaaccgaagaccc

SEQ ID NO: 82 - DNA, 51 bp, synthetic construct
  misc_feature 1..51: note = Primer
  modified_base 38: mod_base = OTHER; note = Deoxyuridine
  source 1..51: mol_type = other DNA
  misc_feature <1: note = 5SpC3 C3 spacer
aaaaaaaaaaaaaaaaaaaaaaaaaaaaaaggcggcangaaccgaagaccc

SEQ ID NO: 83 - DNA, 119 bp, synthetic construct
  misc_feature 1..119: note = Primer
  misc_feature 81..85: note = n is a, c, g, or t
  source 1..119: mol_type = other DNA
ggcggcatgaaccgaaggcccatcctcactatcatcacactggaggactccaggtcaggaaccacttgccaccctgtacannnnnagatcggaagagcacacgtctgaactccagtcac

SEQ ID NO: 84 - DNA, 118 bp, synthetic construct
  misc_feature 1..118: note = Primer
  misc_feature 34..38: note = n is a, c, g, or t
  source 1..118: mol_type = other DNA
acactctttccctacacgacgctcttccgatctnnnnntggcctcaccttgggcctgtgtcatctcctaggttggttctgactgtaccactatccactacaactatatgtgtaacagt

SEQ ID NO: 85 - DNA, 35 bp, synthetic construct
  misc_feature 1..35: note = Primer
  modified_base 12: mod_base = OTHER; note = Deoxyuridine
  modified_base 23: mod_base = OTHER; note = Deoxyuridine
  source 1..35: mol_type = other DNA
actgttacacanatagttgtagnggatagtggtac

SEQ ID NO: 86 - DNA, 65 bp, synthetic construct
  misc_feature 1..65: note = Primer
  misc_feature 42: note = N at position 42 is Deoxyuridine
  modified_base 53: mod_base = OTHER; note = Deoxyuridine
  source 1..65: mol_type = other DNA
  misc_feature <1: note = 5SpC3 C3 spacer
aaaaaaaaaaaaaaaaaaaaaaaaaaaaaaactgttacacanatagttgtagnggatagtggtac

SEQ ID NO: 87 - DNA, 21 bp, synthetic construct
  misc_feature 1..21: note = Primer
  modified_base 9: mod_base = OTHER; note = Deoxyuridine
  source 1..21: mol_type = other DNA
agagaccgncgcacggaggaa

SEQ ID NO: 88 - DNA, 51 bp, synthetic construct
  misc_feature 1..51: note = Primer
  modified_base 39: mod_base = OTHER; note = Deoxyuridine
  source 1..51: mol_type = other DNA
  misc_feature <1: note = 5SpC3 C3 spacer
aaaaaaaaaaaaaaaaaaaaaaaaaaaaaaagagaccgncgcacggaggaa

SEQ ID NO: 89 - DNA, 119 bp, synthetic construct
  misc_feature 1..119: note = Primer
  modified_base 9: mod_base = OTHER; note = Deoxyuridine
  misc_feature 81..85: note = n is a, c, g, or t
  source 1..119: mol_type = other DNA
agagaccgncgcacggaggaagagaatcttcgcaagaaaggagaacctcaccacgagctacccccagggagcaccaagcgnnnnnagatcggaagagcacacgtctgaactccagtcac

SEQ ID NO: 90 - DNA, 118 bp, synthetic construct
  misc_feature 1..118: note = Primer
  misc_feature 34..38: note = n is a, c, g, or t
  source 1..118: mol_type = other DNA
acactctttccctacacgacgctcttccgatctnnnnnttactgcttcttgcttctcttctcctatcctgagtaatggtaatctactggaacggaacagctttgaagtgcgtgtttgt

SEQ ID NO: 91 - DNA, 26 bp, synthetic construct
  misc_feature 1..26: note = Primer
  modified_base 13: mod_base = OTHER; note = Deoxyuridine
  modified_base 21: mod_base = OTHER; note = Deoxyuridine
  source 1..26: mol_type = other DNA
acaaacacgcacntcaaagcngttcc

SEQ ID NO: 92 - DNA, 56 bp, synthetic construct
  misc_feature 1..56: note = Primer
  modified_base 43: mod_base = OTHER; note = Deoxyuridine
  modified_base 51: mod_base = OTHER; note = Deoxyuridine
  source 1..56: mol_type = other DNA
  misc_feature <1: note = 5SpC3 C3 spacer
aaaaaaaaaaaaaaaaaaaaaaaaaaaaaaacaaacacgcacntcaaagcngttcc

SEQ ID NO: 93 - DNA, 34 bp, synthetic construct
  misc_feature 1..34: note = Primer
  modified_base 30: mod_base = OTHER; note = ribouridine
  source 1..34: mol_type = other DNA
  misc_feature >34: note = 3SpC3 C3 spacer
  misc_feature 17^18: note = Internal Dideoxyribose dSpacer
aaggcctgctgaaaatgctgaatataaacntgta

SEQ ID NO: 94 - DNA, 36 bp, synthetic construct
  misc_feature 1..36: note = Primer
  modified_base 32: mod_base = OTHER; note = riboguanosine
  source 1..36: mol_type = other DNA
  misc_feature >36: note = 3SpC3 C3 spacer
  misc_feature 17^18: note = Internal Dideoxyribose dSpacer
cgtccacaaaatgattcgaattagctgtatcntcag

SEQ ID NO: 95 - DNA, 39 bp, synthetic construct
  misc_feature 1..39: note = Primer
  modified_base 35: mod_base = OTHER; note = riboadenosine
  source 1..39: mol_type = other DNA
  misc_feature >39: note = 3SpC3 C3 spacer
  misc_feature 20^21: note = Internal Dideoxyribose dSpacer
tcagatatatttcttcatgagacctcacagtaaanataa

SEQ ID NO: 96 - DNA, 33 bp, synthetic construct
  misc_feature 1..33: note = Primer
  modified_base 29: mod_base = OTHER; note = ribouridine
  source 1..33: mol_type = other DNA
  misc_feature >33: note = 3SpC3 C3 spacer
  misc_feature 15^16: note = Internal Dideoxyribose dSpacer
acaaaatggatccagcaactgttcaaacngata

SEQ ID NO: 97 - DNA, 30 bp, synthetic construct
  misc_feature 1..30: note = Primer
  modified_base 26: mod_base = OTHER; note = riboadenosine
  source 1..30: mol_type = other DNA
  misc_feature >30: note = 3SpC3 C3 spacer
  misc_feature 13^14: note = Internal Dideoxyribose dSpacer
cgccatggccatcacaagcagtcacngcat

SEQ ID NO: 98 - DNA, 29 bp, synthetic construct
  misc_feature 1..29: note = Primer
  modified_base 25: mod_base = OTHER; note = riboguanosine
  source 1..29: mol_type = other DNA
  misc_feature >29: note = 3SpC3 C3 spacer
  misc_feature 13^14: note = Internal Dideoxyribose dSpacer
gctgctcaccatcctatctgagcancgca

SEQ ID NO: 99 - DNA, 32 bp, synthetic construct
  misc_feature 1..32: note = Primer
  modified_base 28: mod_base = OTHER; note = riboadenosine
  source 1..32: mol_type = other DNA
  misc_feature >32: note = 3SpC3 C3 spacer
  misc_feature 16^17: note = Internal Dideoxyribose dSpacer
cttcctacagtactccctgccctcaacnagac

SEQ ID NO: 100 - DNA, 29 bp, synthetic construct
  misc_feature 1..29: note = Primer
  modified_base 25: mod_base = OTHER; note = riboguanosine
  source 1..29: mol_type = other DNA
  misc_feature >29: note = 3SpC3 C3 spacer
  misc_feature 12^13: note = Internal Dideoxyribose dSpacer
ggcggaggtgtgaatcaacccacanctgt

SEQ ID NO: 101 - DNA, 33 bp, synthetic construct
  misc_feature 1..33: note = Primer
  modified_base 29: mod_base = OTHER; note = ribouridine
  source 1..33: mol_type = other DNA
  misc_feature >33: note = 3SpC3 C3 spacer
  misc_feature 15^16: note = Internal Dideoxyribose dSpacer
cctcagcatcttatcgagtggaaggaaanttgt

SEQ ID NO: 102 - DNA, 24 bp, synthetic construct
  misc_feature 1..24: note = Primer
  modified_base 20: mod_base = OTHER; note = ribocytosine
  source 1..24: mol_type = other DNA
  misc_feature >24: note = 3SpC3 C3 spacer
  misc_feature 12^13: note = Internal Dideoxyribose dSpacer
cggctcatagggaccaccanactg

SEQ ID NO: 103 - DNA, 35 bp, synthetic construct
  misc_feature 1..35: note = Primer
  modified_base 31: mod_base = OTHER; note = riboadenosine
  source 1..35: mol_type = other DNA
  misc_feature >35: note = 3SpC3 C3 spacer
  misc_feature 17^18: note = Internal Dideoxyribose dSpacer
ctctgactgtaccaccaccactacaactacntgta

SEQ ID NO: 104 - DNA, 31 bp, synthetic construct
  misc_feature 1..31: note = Primer
  modified_base 27: mod_base = OTHER; note = ribouridine
  source 1..31: mol_type = other DNA
  misc_feature >31: note = 3SpC3 C3 spacer
  misc_feature 15^16: note = Internal Dideoxyribose dSpacer
ctgacctggagtcttcagtgtgatganggta

SEQ ID NO: 105 - DNA, 33 bp, synthetic construct
  misc_feature 1..33: note = Primer
  modified_base 29: mod_base = OTHER; note = riboadenosine
  source 1..33: mol_type = other DNA
  misc_feature >33: note = 3SpC3 C3 spacer
  misc_feature 19^20: note = Internal Dideoxyribose dSpacer
tgagtagtggtaatctactggacggaacngctc

SEQ ID NO: 106 - DNA, 32 bp, synthetic construct
  misc_feature 1..32: note = Primer
  modified_base 28: mod_base = OTHER; note = ribocytosine
  source 1..32: mol_type = other DNA
  misc_feature >32: note = 3SpC3 C3 spacer
  misc_feature 14^15: note = Internal Dideoxyribose dSpacer
gctcccctttcttgggagattctcttcntcta

SEQ ID NO: 107 - DNA, 70 bp, synthetic construct
  misc_feature 1..70: note = KRAS top strand capture oligo
  source 1..70: mol_type = other DNA
ttttttttttgctggtggcgtaggcaagagtgccttgacgatacagctaattcagaatcattttgtggac

SEQ ID NO: 108 - DNA, 70 bp, synthetic construct
  misc_feature 1..70: note = KRAS bottom strand capture oligo
  source 1..70: mol_type = other DNA
ttttttttttacgccaccagctccaactaccacaagtttatattcagtcattttcagcaggccttataat

SEQ ID NO: 109 - DNA, 70 bp, synthetic construct
  misc_feature 1..70: note = BRAF top strand capture oligo
  source 1..70: mol_type = other DNA
ttttttttttgctacagtgaaatctcgatggagtgggtcccatcagtttgaacagttgtctggatccatt

SEQ ID NO: 110 - DNA, 70 bp, synthetic construct
  misc_feature 1..70: note = BRAF bottom strand capture oligo
  source 1..70: mol_type = other DNA
ttttttttttgatttcactgtagctagaccaaaatcacctatttttactgtgaggtcttcatgaagaaat

SEQ ID NO: 111 - DNA, 70 bp, synthetic construct
  misc_feature 1..70: note = TP53 Exon 5.1 top strand capture oligo
  source 1..70: mol_type = other DNA
ttttttttttaagacctgccctgtgcagctgtgggttgattccacacccccgcccggcacccgcgtccgc

SEQ ID NO: 112 - DNA, 70 bp, synthetic construct
  misc_feature 1..70: note = TP53 Exon 5.1 bottom strand capture oligo
  source 1..70: mol_type = other DNA
ttttttttttcacagggcaggtcttggccagttggcaaaacatcttgttgagggcaggagagtactgtag

SEQ ID NO: 113 - DNA, 70 bp, synthetic construct
  misc_feature 1..70: note = TP53 Exon 5.2 top strand capture oligo
  source 1..70: mol_type = other DNA
ttttttttttaggcgctgcccccaccatgagcgctgctcagatagcgatggtgagcagctggagctggag

SEQ ID NO: 114 - DNA, 70 bp, synthetic construct
  misc_feature 1..70: note = TP53 Exon 5.2 bottom strand capture oligo
  source 1..70: mol_type = other DNA
ttttttttttgggcagcgcctcacaacctccgtcatgtgctgtgactgcttgtagatggccatggcgcgg

SEQ ID NO: 115 - DNA, 70 bp, synthetic construct
  misc_feature 1..70: note = TP53 Exon 6 top strand capture oligo
  source 1..70: mol_type = other DNA
ttttttttttttggatgacagaaacacttttcgacatagtgtggtggtgccctatgagccgcctgaggtc

SEQ ID NO: 116 - DNA, 70 bp, synthetic construct
  misc_feature 1..70: note = TP53 Exon 6 bottom strand capture oligo
  source 1..70: mol_type = other DNA
ttttttttttgtcatccaaatactccacacgcaaatttccttccactcggataagatgctgaggaggagc

SEQ ID NO: 117 - DNA, 70 bp, synthetic construct
  misc_feature 1..70: note = TP53 Exon 7 top strand capture oligo
  source 1..70: mol_type = other DNA
ttttttttttggcggcatgaaccggaggcccatcctcaccatcatcacactggaagactccaggtcagga

SEQ ID NO: 118 - DNA, 70 bp, synthetic construct
  misc_feature 1..70: note = TP53 Exon 7 bottom strand capture oligo
  source 1..70: mol_type = other DNA
ttttttttttcatgccgcccatgcaggaactgttacacatgtagttgtagtggatggtggtacagtcaga

SEQ ID NO: 119 - DNA, 70 bp, synthetic construct
  misc_feature 1..70: note = TP53 Exon 8 top strand capture oligo
  source 1..70: mol_type = other DNA
tttttttttttgtcctgggagagaccgacgcacagaggaagagaatctccgcaagaaaggagagcctcac

SEQ ID NO: 120 - DNA, 70 bp, synthetic construct
  misc_feature 1..70: note = TP53 Exon 8 bottom strand capture oligo
  source 1..70: mol_type = other DNA
ttttttttttcccaggacatgcacaaacacgcacctcaaagctgttccgtcccagtagattaccactact

SEQ ID NO: 121 - DNA, 42 bp, synthetic construct
  misc_feature 1..42: note = Blunt end linker
  modified_base 6: mod_base = OTHER; note = Deoxyuridine
  modified_base 12: mod_base = OTHER; note = Deoxyuridine
  modified_base 21: mod_base = OTHER; note = Deoxyuridine
  misc_feature 35..39: note = n is a, c, g, or t
  source 1..42: mol_type = other DNA
  misc_feature 22..23: note = thiophosphate backbone
gtgacnggagtncagacgtgngctcttccgatctnnnnngcc

SEQ ID NO: 122 - DNA, 21 bp, synthetic construct
  misc_feature 1..21: note = Blunt end linker
  modified_base 4..8: mod_base = OTHER; note = 5-nitroindole
  modified_base 12: mod_base = OTHER; note = Deoxyuridine
  source 1..21: mol_type = other DNA
  misc_feature >21: note = 3SpC3 C3 spacer
ggcnnnnnagancggaagagc

SEQ ID NO: 123 - DNA, 27 bp, synthetic construct
  misc_feature 1..27: note = Primer
  modified_base 4: mod_base = OTHER; note = Deoxyuridine
  modified_base 15: mod_base = OTHER; note = Deoxyuridine
  source 1..27: mol_type = other DNA
agancggaagagcgncgtgtagggaaa

SEQ ID NO: 124 - DNA, 57 bp, synthetic construct
  misc_feature 1..57: note = Primer
  modified_base 34: mod_base = OTHER; note = Deoxyuridine
  modified_base 45: mod_base = OTHER; note = Deoxyuridine
  source 1..57: mol_type = other DNA
  misc_feature <1: note = 5SpC3 C3 spacer
aaaaaaaaaaaaaaaaaaaaaaaaaaaaaaagancggaagagcgncgtgtagggaaa

SEQ ID NO: 125 - DNA, 92 bp, synthetic construct
  misc_feature 1..92: note = Primer
  modified_base 4: mod_base = OTHER; note = Deoxyuridine
  modified_base 15: mod_base = OTHER; note = Deoxyuridine
  modified_base 31: mod_base = OTHER; note = Deoxyuridine
  modified_base 49: mod_base = OTHER; note = Deoxyuridine
  modified_base 64: mod_base = OTHER; note = Deoxyuridine
  modified_base 80: mod_base = OTHER; note = Deoxyuridine
  source 1..92: mol_type = other DNA
agancggaagagcgncgtgtagggaaagagngtaggatagggtgtaganctcggtggtcgccgnatcattgcgagtgtgncaagcagaagac

SEQ ID NO: 126 - DNA, 82 bp, synthetic construct
  misc_feature 1..82: note = Primer
  modified_base 19: mod_base = OTHER; note = Deoxyuridine
  modified_base 31: mod_base = OTHER; note = Deoxyuridine
  modified_base 49: mod_base = OTHER; note = Deoxyuridine
  modified_base 65: mod_base = OTHER; note = Deoxyuridine
  source 1..82: mol_type = other DNA
aaaaaggaagagcacacgnctgaactccagncaccgagtaatatctcgnatgccgtcttctgctngacacactcgcaatgat

SEQ ID NO: 127 - DNA, 27 bp, synthetic construct
  misc_feature 1..27: note = Primer
  modified_base 19: mod_base = OTHER; note = Deoxyuridine
  source 1..27: mol_type = other DNA
aaaaaggaagagcacacgnctgaactc

SEQ ID NO: 128 - DNA, 52 bp, synthetic construct
  misc_feature 1..52: note = Primer
  modified_base 44: mod_base = OTHER; note = Deoxyuridine
  source 1..52: mol_type = other DNA
  misc_feature <1: note = 5SpC3 C3 spacer
aaaaaaaaaaaaaaaaaaaaaaaaaaaaaaggaagagcacacgnctgaactc

SEQ ID NO: 129 - DNA, 84 bp, synthetic construct
  misc_feature 1..84: note = Long D702 blunt end Linker
  modified_base 10: mod_base = OTHER; note = Deoxyuridine
  modified_base 27: mod_base = OTHER; note = Deoxyuridine
  modified_base 35: mod_base = OTHER; note = Deoxyuridine
  modified_base 48: mod_base = OTHER; note = Deoxyuridine
  modified_base 54: mod_base = OTHER; note = Deoxyuridine
  modified_base 63: mod_base = OTHER; note = Deoxyuridine
  misc_feature 77..81: note = n is a, c, g, or t
  source 1..84: mol_type = other DNA
  misc_feature 64..65: note = thiophosphate backbone
gcgagtgtgncaagcagaagacggcanacgagatnccggagagtgacnggagtncagacgtgngctcttccgatctnnnnngcc

SEQ ID NO: 130 - DNA, 100 bp, synthetic construct
  misc_feature 1..100: note = Primer
  modified_base 18: mod_base = OTHER; note = Deoxyuridine
  modified_base 33: mod_base = OTHER; note = Deoxyuridine
  modified_base 51: mod_base = OTHER; note = Deoxyuridine
  modified_base 64: mod_base = OTHER; note = Deoxyuridine
  modified_base 80: mod_base = OTHER; note = Deoxyuridine
  modified_base 96: mod_base = OTHER; note = Deoxyuridine
  source 1..100: mol_type = other DNA
agatcggaagagcgtcgngtagggaaagagtgnaggatagggtgtagatcncggtggtcgccgnatcattgcgagtgtgncaagcagaagacggcntttt

SEQ ID NO: 131 - DNA, 70 bp, synthetic construct
  misc_feature 1..70: note = D503 thiophosphate Linker
  source 1..70: mol_type = other DNA
  misc_feature 2..3: note = thiophosphate backbone
aatgatacggcgaccaccgagatctacaccctatcctacactctttccctacacgacgctcttccgatct

SEQ ID NO: 132 - DNA, 65 bp, synthetic construct
  misc_feature 1..65: note = D707 Linker
  source 1..65: mol_type = other DNA
gatcggaagagcacacgtctgaactccagtcacagcttcagatctcgtatgccgtcttctgcttg

SEQ ID NO: 133 - DNA, 67 bp, synthetic construct
  misc_feature 1..67: note = Universal reverse linker bridge
  modified_base 9: mod_base = OTHER; note = Deoxyuridine
  modified_base 22: mod_base = OTHER; note = Deoxyuridine
  modified_base 38: mod_base = OTHER; note = Deoxyuridine
  modified_base 55: mod_base = OTHER; note = Deoxyuridine
  source 1..67: mol_type = other DNA
tgtagatcncggtggtcgccgnatcattgcgagtgtgncaagcagaagacggcanacgagatttttt

SEQ ID NO: 134 - DNA, 70 bp, synthetic construct
  misc_feature 1..70: note = D504 thiophosphate Linker
  source 1..70: mol_type = other DNA
  misc_feature 2..3: note = thiophosphate backbone
aatgatacggcgaccaccgagatctacacggctctgaacactctttccctacacgacgctcttccgatct

SEQ ID NO: 135 - DNA, 11 bp, synthetic construct
  misc_feature 1..11: note = Small 5'-phos Linker
  source 1..11: mol_type = other DNA
cctccgaccgt

SEQ ID NO: 136 - DNA, 82 bp, synthetic construct
  misc_feature 1..82: note = D708 modified Linker
  misc_feature 11..16: note = n is a, c, g, or t
  source 1..82: mol_type = other DNA
cggtcggaggnnnnnnagatcggaagagcacacgtctgaactccagtcacgcgcattaatctcgtatgccgtcttctgcttg

SEQ ID NO: 137 - DNA, 70 bp, synthetic construct
  misc_feature 1..70: note = D505 thiophosphate Linker
  source 1..70: mol_type = other DNA
  misc_feature 2..3: note = thiophosphate backbone
aatgatacggcgaccaccgagatctacacaggcgaagacactctttccctacacgacgctcttccgatct

SEQ ID NO: 138 - skipped

SEQ ID NO: 139 - DNA, 79 bp, synthetic construct
  misc_feature 1..79: note = D506 - 2rG-LNA Linker
  misc_feature 71..76: note = n is a, c, g, or t
  modified_base 77..78: mod_base = OTHER; note = riboguanosine
  modified_base 79: mod_base = OTHER; note = locked nucleic acid guanosine
  source 1..79: mol_type = other DNA
  misc_feature 2..3: note = thiophosphate backbone
aatgatacggcgaccaccgagatctacactaatcttaacactctttccctacacgacgctcttccgatctnnnnnnnnn

SEQ ID NO: 140 - DNA, 65 bp, synthetic construct
  misc_feature 1..65: note = D709 Linker
  source 1..65: mol_type = other DNA
gatcggaagagcacacgtctgaactccagtcaccatagccgatctcgtatgccgtcttctgcttg

SEQ ID NO: 141 - DNA, 107 bp, synthetic construct
  misc_feature 1..107: note = Primer
  modified_base 20: mod_base = OTHER; note = Deoxyuridine
  modified_base 40: mod_base = OTHER; note = Deoxyuridine
  modified_base 50: mod_base = OTHER; note = Deoxyuridine
  modified_base 66: mod_base = OTHER; note = Deoxyuridine
  modified_base 80: mod_base = OTHER; note = Deoxyuridine
  modified_base 96: mod_base = OTHER; note = Deoxyuridine
  source 1..107: mol_type = other DNA
  misc_feature 2..3: note = thiophosphate backbone
cgatacagctaattcagaancattttgtggacgaattttnaggtcgccgnatcattgcgagtgtgncaagcagaagacgntttttgctggtggcgnaggcaagagtg

SEQ ID NO: 142 - DNA, 115 bp, synthetic construct
  misc_feature 1..115: note = Primer
  modified_base 27: mod_base = OTHER; note = Deoxyuridine
  modified_base 49: mod_base = OTHER; note = Deoxyuridine
  modified_base 59: mod_base = OTHER; note = Deoxyuridine
  modified_base 75: mod_base = OTHER; note = Deoxyuridine
  modified_base 89: mod_base = OTHER; note = Deoxyuridine
  modified_base 106: mod_base = OTHER; note = Deoxyuridine
  source 1..115: mol_type = other DNA
  misc_feature 2..3: note = thiophosphate backbone
ttatattcagtcattttcagcaggccntataataaaaataatgattttnaggtcgccgnatcattgcgagtgtgncaagcagaagacgntttttacgccaccagcnccaactacc

SEQ ID NO: 143 - DNA, 110 bp, synthetic construct
  misc_feature 1..110: note = Primer
  modified_base 14: mod_base = OTHER; note = Deoxyuridine
  modified_base 20: mod_base = OTHER; note = Deoxyuridine
  modified_base 36: mod_base = OTHER; note = Deoxyuridine
  modified_base 46: mod_base = OTHER; note = Deoxyuridine
  modified_base 62: mod_base = OTHER; note = Deoxyuridine
  modified_base 76: mod_base = OTHER; note = Deoxyuridine
  modified_base 94: mod_base = OTHER; note = Deoxyuridine
  modified_base 100: mod_base = OTHER; note = Deoxyuridine
  source 1..110: mol_type = other DNA
  misc_feature 2..3: note = thiophosphate backbone
gtttgaacagttgnctgganccattttgtggttttnaggtcgccgnatcattgcgagtgtgncaagcagaagacgntttttgctacagtgaaanctcganggagtgggtc

SEQ ID NO: 144 - DNA, 130 bp, synthetic construct
  misc_feature 1..130: note = Primer
  modified_base 16: mod_base = OTHER; note = Deoxyuridine
  modified_base 29: mod_base = OTHER; note = Deoxyuridine
  modified_base 47: mod_base = OTHER; note = Deoxyuridine
  modified_base 57: mod_base = OTHER; note = Deoxyuridine
  modified_base 73: mod_base = OTHER; note = Deoxyuridine
  modified_base 87: mod_base = OTHER; note = Deoxyuridine
  modified_base 107: mod_base = OTHER; note = Deoxyuridine
  source 1..130: mol_type = other DNA
  misc_feature 2..3: note = thiophosphate backbone
gtcttcatgaagaaanatatctgaggtgnagtaagtaaaggattttnaggtcgccgnatcattgcgagtgtgncaagcagaagacgntttttgatttcactgtagcnagaccaaaatcacctatttttac

SEQ ID NO: 145 - DNA, 92 bp, synthetic construct
  misc_feature 1..92: note = Primer
  modified_base 13: mod_base = OTHER; note = Deoxyuridine
  modified_base 24: mod_base = OTHER; note = Deoxyuridine
  modified_base 34: mod_base = OTHER; note = Deoxyuridine
  modified_base 50: mod_base = OTHER; note = Deoxyuridine
  modified_base 64: mod_base = OTHER; note = Deoxyuridine
  modified_base 76: mod_base = OTHER; note = Deoxyuridine
  source 1..92: mol_type = other DNA
  misc_feature 2..3: note = thiophosphate backbone
tgattccacaccnccgcccttttnaggtcgccgnatcattgcgagtgtgncaagcagaagacgntttttaagaccngccctgtgcagctgtg

SEQ ID NO: 146 - DNA, 104 bp, synthetic construct
  misc_feature 1..104: note = Primer
  modified_base 15: mod_base = OTHER; note = Deoxyuridine
  modified_base 35: mod_base = OTHER; note = Deoxyuridine
  modified_base 45: mod_base = OTHER; note = Deoxyuridine
  modified_base 61: mod_base = OTHER; note = Deoxyuridine
  modified_base 75: mod_base = OTHER; note = Deoxyuridine
  modified_base 88: mod_base = OTHER; note = Deoxyuridine
  source 1..104: mol_type = other DNA
  misc_feature 2..3: note = thiophosphate backbone
catcttgttgagggnaggagagtactgtagttttnaggtcgccgnatcattgcgagtgtgncaagcagaagacgntttttcacagggnaggtcttggccagttg

SEQ ID NO: 147 - DNA, 95 bp, synthetic construct
  misc_feature 1..95: note = Primer
  modified_base 17: mod_base = OTHER; note = Deoxyuridine
  modified_base 31: mod_base = OTHER; note = Deoxyuridine
  modified_base 41: mod_base = OTHER; note = Deoxyuridine
  modified_base 57: mod_base = OTHER; note = Deoxyuridine
  modified_base 71: mod_base = OTHER; note = Deoxyuridine
  modified_base 83: mod_base = OTHER; note = Deoxyuridine
  source 1..95: mol_type = other DNA
  misc_feature 2..3: note = thiophosphate backbone
gctcagatagcgatggngagcagctgttttnaggtcgccgnatcattgcgagtgtgncaagcagaagacgntttttaggcgcngcccccaccatg

SEQ ID NO: 148 - DNA, 96 bp, synthetic construct
  misc_feature 1..96: note = Primer
  modified_base 21: mod_base = OTHER; note = Deoxyuridine
  modified_base 31: mod_base = OTHER; note = Deoxyuridine
  modified_base 41: mod_base = OTHER; note = Deoxyuridine
  modified_base 57: mod_base = OTHER; note = Deoxyuridine
  modified_base 71: mod_base = OTHER; note = Deoxyuridine
  modified_base 80: mod_base = OTHER; note = Deoxyuridine
  source 1..96: mol_type = other DNA
  misc_feature 2..3: note = thiophosphate backbone
gtgctgtgactgcttgtaganggccattttnaggtcgccgnatcattgcgagtgtgncaagcagaagacgntttttgggnagcgcctcacaacctc

SEQ ID NO: 149 - DNA, 105 bp, synthetic construct
  misc_feature 1..105: note = Primer
  modified_base 15: mod_base = OTHER; note = Deoxyuridine
  modified_base 27: mod_base = OTHER; note = Deoxyuridine
  modified_base 37: mod_base = OTHER; note = Deoxyuridine
  modified_base 53: mod_base = OTHER; note = Deoxyuridine
  modified_base 67: mod_base = OTHER; note = Deoxyuridine
  modified_base 78: mod_base = OTHER; note = Deoxyuridine
  source 1..105: mol_type = other DNA
  misc_feature 2..3: note = thiophosphate backbone
ccctatgagccgccngaggtctttttnaggtcgccgnatcattgcgagtgtgncaagcagaagacgntttttttggangacagaaacacttttcgacatagtgtg

SEQ ID NO: 150 - DNA, 107 bp, synthetic construct
  misc_feature 1..107: note = Primer
  modified_base 22: mod_base = OTHER; note = Deoxyuridine
  modified_base 32: mod_base = OTHER; note = Deoxyuridine
  modified_base 42: mod_base = OTHER; note = Deoxyuridine
  modified_base 58: mod_base = OTHER; note = Deoxyuridine
  modified_base 72: mod_base = OTHER; note = Deoxyuridine
  modified_base 88: mod_base = OTHER; note = Deoxyuridine
  source 1..107: mol_type = other DNA
  misc_feature 2..3: note = thiophosphate backbone
tcggataagatgctgaggaggngccagttttnaggtcgccgnatcattgcgagtgtgncaagcagaagacgntttttgtcatccaaanactccacacgcaaatttcc

SEQ ID NO: 151 - DNA, 98 bp, synthetic construct
  misc_feature 1..98: note = Primer
  modified_base 22: mod_base = OTHER; note = Deoxyuridine
  modified_base 32: mod_base = OTHER; note = Deoxyuridine
  modified_base 42: mod_base = OTHER; note = Deoxyuridine
  modified_base 58: mod_base = OTHER; note = Deoxyuridine
  modified_base 72: mod_base = OTHER; note = Deoxyuridine
  modified_base 85: mod_base = OTHER; note = Deoxyuridine
  source 1..98: mol_type = other DNA
  misc_feature 2..3: note = thiophosphate backbone
accatcatcacactggaagacnccaggttttnaggtcgccgnatcattgcgagtgtgncaagcagaagacgntttttggcggcangaaccggagaccc

SEQ ID NO: 152 - DNA, 103 bp, synthetic construct
  misc_feature 1..103: note = Primer
  modified_base 23: mod_base = OTHER; note = Deoxyuridine
  modified_base 36: mod_base = OTHER; note = Deoxyuridine
  modified_base 46: mod_base = OTHER; note = Deoxyuridine
  modified_base 62: mod_base = OTHER; note = Deoxyuridine
  modified_base 76: mod_base = OTHER; note = Deoxyuridine
  modified_base 86: mod_base = OTHER; note = Deoxyuridine
  source 1..103: mol_type = other DNA
  misc_feature 2..3: note = thiophosphate backbone
atgtagttgtagtggatggtggnacagtcagttttnaggtcgccgnatcattgcgagtgtgncaagcagaagacgntttttcatgncgcccatgcaggaactg

SEQ ID NO: 153 - DNA, 99 bp, synthetic construct
  misc_feature 1..99: note = Primer
  modified_base 25: mod_base = OTHER; note = Deoxyuridine
  modified_base 34: mod_base = OTHER; note = Deoxyuridine
  modified_base 44: mod_base = OTHER; note = Deoxyuridine
  modified_base 60: mod_base = OTHER; note = Deoxyuridine
  modified_base 74: mod_base = OTHER; note = Deoxyuridine
  modified_base 85: mod_base = OTHER; note = Deoxyuridine
  source 1..99: mol_type = other DNA
  misc_feature 2..3: note = thiophosphate backbone
ggaagagaatctccgcaagaaaggngagcttttnaggtcgccgnatcattgcgagtgtgncaagcagaagacgnttttttgtccngggagagaccggcg

SEQ ID NO: 154 - DNA, 107 bp, synthetic construct
  misc_feature 1..107: note = Primer
  modified_base 17: mod_base = OTHER; note = Deoxyuridine
  modified_base 35: mod_base = OTHER; note = Deoxyuridine
  modified_base 45: mod_base = OTHER; note = Deoxyuridine
  modified_base 61: mod_base = OTHER; note = Deoxyuridine
  modified_base 75: mod_base = OTHER; note = Deoxyuridine
  modified_base 90: mod_base = OTHER; note = Deoxyuridine
  source 1..107: mol_type = other DNA
  misc_feature 2..3: note = thiophosphate backbone
gttccgtcccagtagantaccactactcagttttnaggtcgccgnatcattgcgagtgtgncaagcagaagacgntttttcccaggacangcacaaacacgcacctc

SEQ ID NO: 155 - DNA, 13 bp, synthetic construct
  source 1..13: mol_type = other DNA
  modified_base 7: mod_base = OTHER; note = n is selected from deoxyinosine, deoxyguanosine, deoxyadenosine, and deoxythymidine
  misc_feature 1..13: note = Miniduplex
ggaaaanaaaagg

SEQ ID NO: 156 - DNA, 13 bp, synthetic construct
  source 1..13: mol_type = other DNA
  modified_base 7: mod_base = OTHER; note = n is deoxycytidine, deoxyadenosine, deoxyguanosine, deoxythymidine, or deoxyuridine
  misc_feature 1..13: note = Heteroduplex
ccttttnttttcc

SEQ ID NO: 157 - DNA, 12 bp, synthetic construct
  source 1..12: mol_type = other DNA
  misc_feature 1..12: note = Self-complimentary
  modified_base 6: mod_base = OTHER; note = n is selected from deoxyinosine, deoxyguanosine, deoxyadenosine, and deoxythymidine
  modified_base 7: mod_base = OTHER; note = n is deoxycytidine, deoxyadenosine, deoxyguanosine, deoxythymidine, or deoxyuridine
gggaannttccc